European Patent Specification EP 4 010 493 B1, published December 18, 2024. Title: Methods for the multiplexed isothermal amplification of nucleic acid sequences. Applicant: DNAE DIAGNOSTICS LTD. The sequence listing filed with the application follows.

SEQUENCE LISTING (27 sequences)

SEQ ID NO: 1 - DNA, 46 bp, LAMP_LP1_v1
  T at position 1 has a PO4 at position 5
tccagttatctcgtatgccgtcttctgcttgaactggatctataag

SEQ ID NO: 2 - DNA, 44 bp, LAMP_LP2_v1
gactcctcagctagcgaatgatacggcgaccaccgacgctagct

SEQ ID NO: 3 - DNA, 41 bp, LAMP_LP1_v2
  T at position 1 has a PO4 at position 5
tccagttttcagaggatctagtcggcaactggatctataag

SEQ ID NO: 4 - DNA, 42 bp, LAMP_LP2_v2
gactcctcagctagcgcttggcttcattgtggtccgctagct

SEQ ID NO: 5 - DNA, 58 bp, SHRK_INS01
  G at position 1 has a PO4 at position 5
gaggagtcgctccatcggtgtgtacgcgatggataccggctcaggcgcaacttataga

SEQ ID NO: 6 - DNA, 72 bp, SBL_PHIX_01
  G, A, C and T at positions 1, 2, 3 and 4 are linked by phosphorothioate bonds.
gactcctcagctagcgaatgatacggcgaccaccgacgctagctgaggagtccaatccgtacgtttccagac

SEQ ID NO: 7 - DNA, 74 bp, SBL_PHIX_02
cttatagatccagttcaagcagaagacggcatacgagataactggatctataagacggcagcaataaactcaac

SEQ ID NO: 8 - DNA, 72 bp, SBL_PHIX_03
  G, A, C and T at positions 1, 2, 3 and 4 are linked by phosphorothioate bonds.
gactcctcagctagcgaatgatacggcgaccaccgacgctagctgaggagtcttaaagccgctgaattgttc

SEQ ID NO: 9 - DNA, 74 bp, SBL_PHIX_04
cttatagatccagttcaagcagaagacggcatacgagataactggatctataagtgcctttagtacctcgcaac

SEQ ID NO: 10 - DNA, 72 bp, SBL_PHIX_05
  G, A, C and T at positions 1, 2, 3 and 4 are linked by phosphorothioate bonds.
gactcctcagctagcgaatgatacggcgaccaccgacgctagctgaggagtccgcctactgcgactaaagag

SEQ ID NO: 11 - DNA, 78 bp, SBL_PHIX_06
cttatagatccagttcaagcagaagacggcatacgagataactggatctataagaacgataccactgactgaccctca

SEQ ID NO: 12 - DNA, 72 bp, SBL_PHIX_07
  G, A, C and T at positions 1, 2, 3 and 4 are linked by phosphorothioate bonds.
gactcctcagctagcgaatgatacggcgaccaccgacgctagctgaggagtccttcttcggcacctgtttta

SEQ ID NO: 13 - DNA, 74 bp, SBL_PHIX_08
cttatagatccagttcaagcagaagacggcatacgagataactggatctataagaaaaatttagggtcggcatc

SEQ ID NO: 14 - DNA, 72 bp, SBL_PHIX_09
  G, A, C and T at positions 1, 2, 3 and 4 are linked by phosphorothioate bonds.
gactcctcagctagcgaatgatacggcgaccaccgacgctagctgaggagtctcaaggtgatgtgcttgcta

SEQ ID NO: 15 - DNA, 74 bp, SBL_PHIX_10
cttatagatccagttcaagcagaagacggcatacgagataactggatctataagccaagtccaaccaaatcaag

SEQ ID NO: 16 - DNA, 148 bp, LAMP_T01_v1
gactcctcagctagcgaatgatacggcgaccaccgacgctagctgaggagtcgctccatcggtgtgtacgcgatggataccggctcaggcgcaacttatagatccagttatctcgtatgccgtcttctgcttgaactggatctataag

SEQ ID NO: 17 - DNA, 37 bp, LP1rc_INV_v1
  C, G, A and G at positions 34, 35, 36 and 37 are linked by phosphorothioate bonds.
cttatagatccagttcaagcagaagacggcatacgag

SEQ ID NO: 18 - DNA, 33 bp, LP2_INV_v1
  C, C, A and C at positions 30, 31, 32 and 33 are linked by phosphorothioate bonds.
gactcctcagctagcgaatgatacggcgaccac

SEQ ID NO: 19 - DNA, 32 bp, LP1rc_INV_v2
  T, C, T and G at positions 29, 30, 31 and 32 are linked by phosphorothioate bonds.
cttatagatccagttgccgactagatcctctg

SEQ ID NO: 20 - DNA, 32 bp, LP2_INV_v2
  G, T, G and G at positions 29, 30, 31 and 32 are linked by phosphorothioate bonds.
gactcctcagctagcgcttggcttcattgtgg

SEQ ID NO: 21 - DNA, 97 bp, SBL_T01
gaggagtctcgccttcgtatagcctattactcgcgtctaatggctctgagagattcctcgccttaaggcgaagattcagaaactgcatacttataga

SEQ ID NO: 22 - DNA, 97 bp, SBL_T02
gaggagtctatcctccgtaatcttagaattcgtgtagagagatagaggcattactcgttatgcgacaggacgtctgaagctgtagagagcttataga

SEQ ID NO: 23 - DNA, 97 bp, SBL_T03
gaggagtcctagtaccggtactgactaatgcgctcgactagtatagcctcggctatgttctgcctcctatcctcgctcattcgtctaatcttataga

SEQ ID NO: 24 - DNA, 97 bp, SBL_T04
gaggagtcgtaaggacgtatagcctattactcgcagcctcgatagaggcattactcgtatcctctatagaggctccgcgaacagcctcgcttataga

SEQ ID NO: 25 - DNA, 97 bp, SBL_T05
gaggagtcttctgcccgcctatccttctcgcgccctagagtatagaggcattactcgtggagtcccctatcctcgctcatttcgactagcttataga

SEQ ID NO: 26 - DNA, 97 bp, SBL_T06
gaggagtcactgcatcgtatagcctattactcgtgcctcttggctctgaagcgatagttaaggagcctatcctcgctcatttgcctcttcttataga

SEQ ID NO: 27 - DNA, 97 bp, SBL_T07
gaggagtcaggagtccgtatagcctattactcggcgtaagaatagaggcattactcgtatgcctacctatcctcgctcattcctagagtcttataga